European Patent Specification EP 4 042 166 B1, published April 9, 2025. Title: Compositions and Methods for an IL-17 Target Engagement Assay with Small Molecule Modulators. Applicant: Janssen Biotech, Inc. The sequence listing filed with the application follows.

SEQUENCE LISTING (39 sequences)

SEQ ID NO: 1 - protein, 12 aa, Artificial Sequence
  LCDR1 of mAb4538, mAb732, and mAb3584
RASQNVWAFYLA

SEQ ID NO: 2 - protein, 7 aa, Artificial Sequence
  LCDR2 of mAb4538, mAb732, and mAb3584
GASNRAT

SEQ ID NO: 3 - protein, 10 aa, Artificial Sequence
  LCDR3 of mAb4538 and mAb3584
QQYRSTLSLT

SEQ ID NO: 4 - protein, 7 aa, Artificial Sequence
  HCDR1 of mAb4538, mAb732, and mAb3584
SSSAAWG

SEQ ID NO: 5 - protein, 18 aa, Artificial Sequence
  HCDR2 of mAb4538, mAb732, and mAb3584
RISYRSKWYNDYAVSVKS

SEQ ID NO: 6 - protein, 12 aa, Artificial Sequence
  HCDR3 of mAb4538, and mAb732
EVDSMYYSYFDI

SEQ ID NO: 7 - protein, 109 aa, Artificial Sequence
  VL of mAb4538 and mAb3584
EIVLTQSPATLSLSPGERATLSCRASQNVWAFYLAWYQQKPGQAPRLLIYGASNRATGIPARFSGSGSGTDFTLTISSLEPEDFAVYYCQQYRSTLSLTFGQGTKVEIK

SEQ ID NO: 8 - protein, 124 aa, Artificial Sequence
  VH of mAb4538 and mAb732
QVQLQQSGPGLVKPSQTLSLTCAISGDSVSSSSAAWGWIRQSPSRGLEWLGRISYRSKWYNDYAVSVKSRITINPDTSKNQFSLQLNSVTPEDTAVYYCAREVDSMYYSYFDIWGQGTLVTVSS

SEQ ID NO: 9 - protein, 215 aa, Artificial Sequence
  LC of mAb4538 and mAb3584
EIVLTQSPATLSLSPGERATLSCRASQNVWAFYLAWYQQKPGQAPRLLIYGASNRATGIPARFSGSGSGTDFTLTISSLEPEDFAVYYCQQYRSTLSLTFGQGTKVEIKGQPKAAPSVTLFPPSSEELQANKATLVCLISDFYPGAVTVAWKADSSPVKAGVETTTPSKQSNNKYAASSYLSLTPEQWKSHRSYSCQVTHEGSTVEKTVAPTECS

SEQ ID NO: 10 - protein, 454 aa, Artificial Sequence
  HC of mAb4538 and mAb732
QVQLQQSGPGLVKPSQTLSLTCAISGDSVSSSSAAWGWIRQSPSRGLEWLGRISYRSKWYNDYAVSVKSRITINPDTSKNQFSLQLNSVTPEDTAVYYCAREVDSMYYSYFDIWGQGTLVTVSSASTKGPSVFPLAPSSKSTSGGTAALGCLVKDYFPEPVTVSWNSGALTSGVHTFPAVLQSSGLYSLSSVVTVPSSSLGTQTYICNVNHKPSNTKVDKKVEPKSCDKTHTCPPCPAPELLGGPSVFLFPPKPKDTLMISRTPEVTCVVVDVSHEDPEVKFNWYVDGVEVHNAKTKPREEQYNSTYRVVSVLTVLHQDWLNGKEYKCKVSNKALPAPIEKTISKAKGQPREPQVYTLPPSRDELTKNQVSLTCLVKGFYPSDIAVEWESNGQPENNYKTTPPVLDSDGSFFLYSKLTVDKSRWQQGNVFSCSVMHEALHNHYTQKSLSLSPGK

SEQ ID NO: 11 - protein, 10 aa, Artificial Sequence
  LCDR3 of mAb732
TQYYSSPSLT

SEQ ID NO: 12 - protein, 109 aa, Artificial Sequence
  VL of mAb732
EIVLTQSPATLSLSPGERATLSCRASQNVWAFYLAWYQQKPGQAPRLLIYGASNRATGIPARFSGSGSGTDFTLTISSLEPEDFAVYYCTQYYSSPSLTFGQGTKVEIK

SEQ ID NO: 13 - protein, 11 aa, Artificial Sequence
  LCDR1 of mAb7024 and mAb3077
RASQGISNWLN

SEQ ID NO: 14 - protein, 7 aa, Artificial Sequence
  LCDR2 of mAb7024 and mAb3077
AASSLQS

SEQ ID NO: 15 - protein, 8 aa, Artificial Sequence
  LCDR3 of mAb7024 and mAb3077
QQYSDDPT

SEQ ID NO: 16 - protein, 5 aa, Artificial Sequence
  HCDR1 of mAb7024 and mAb3077
SYAIS

SEQ ID NO: 17 - protein, 17 aa, Artificial Sequence
  HCDR2 of mAb7024
SIIPWFGTTNYAQKFQG

SEQ ID NO: 18 - protein, 8 aa, Artificial Sequence
  HCDR3 of mAb7024 and mAb3077
DSEYYFDH

SEQ ID NO: 19 - protein, 106 aa, Artificial Sequence
  VL of mAb7024 and mAb3077
DIQMTQSPSSVSASVGDRVTITCRASQGISNWLNWYQQKPGKAPKLLIYAASSLQSGVPSRFSGSGSGTDFTLTISSLQPEDFATYYCQQYSDDPTFGQGTKVEIK

SEQ ID NO: 20 - protein, 117 aa, Artificial Sequence
  VH of mAb7024
QVQLVQSGAEVKKPGSSVKVSCKASGGTFSSYAISWVRQAPGQGLEWMGSIIPWFGTTNYAQKFQGRVTITADESTSTAYMELSSLRSEDTAVYYCARDSEYYFDHWGQGTLVTVSS

SEQ ID NO: 21 - protein, 212 aa, Artificial Sequence
  LC of mAb7024 and mAb3077
DIQMTQSPSSVSASVGDRVTITCRASQGISNWLNWYQQKPGKAPKLLIYAASSLQSGVPSRFSGSGSGTDFTLTISSLQPEDFATYYCQQYSDDPTFGQGTKVEIKGQPKAAPSVTLFPPSSEELQANKATLVCLISDFYPGAVTVAWKADSSPVKAGVETTTPSKQSNNKYAASSYLSLTPEQWKSHRSYSCQVTHEGSTVEKTVAPTECS

SEQ ID NO: 22 - protein, 447 aa, Artificial Sequence
  HC of mAb3077
QVQLVQSGAEVKKPGSSVKVSCKASGGTFSSYAISWVRQAPGQGLEWMGSIIPWFGWTNYAQKFQGRVTITADESTSTAYMELSSLRSEDTAVYYCARDSEYYFDHWGQGTLVTVSSASTKGPSVFPLAPSSKSTSGGTAALGCLVKDYFPEPVTVSWNSGALTSGVHTFPAVLQSSGLYSLSSVVTVPSSSLGTQTYICNVNHKPSNTKVDKKVEPKSCDKTHTCPPCPAPELLGGPSVFLFPPKPKDTLMISRTPEVTCVVVDVSHEDPEVKFNWYVDGVEVHNAKTKPREEQYNSTYRVVSVLTVLHQDWLNGKEYKCKVSNKALPAPIEKTISKAKGQPREPQVYTLPPSRDELTKNQVSLTCLVKGFYPSDIAVEWESNGQPENNYKTTPPVLDSDGSFFLYSKLTVDKSRWQQGNVFSCSVMHEALHNHYTQKSLSLSPGK

SEQ ID NO: 23 - protein, 11 aa, Artificial Sequence
  LCDR1 of mAb5548
SGDNLGDKYAN

SEQ ID NO: 24 - protein, 7 aa, Artificial Sequence
  LCDR2 of mAb5548
DDIDRPS

SEQ ID NO: 25 - protein, 11 aa, Artificial Sequence
  LCDR3 of mAb5548
GSYDFFLGLIV

SEQ ID NO: 26 - protein, 5 aa, Artificial Sequence
  HCDR1 of mAb5548
SYAMS

SEQ ID NO: 27 - protein, 17 aa, Artificial Sequence
  HCDR2 of mAb5548
TISLTSGFTYYADSVKG

SEQ ID NO: 28 - protein, 6 aa, Artificial Sequence
  HCDR3 of mAb5548
QLTLDV

SEQ ID NO: 29 - protein, 108 aa, Artificial Sequence
  VL of mAb5548
QSVLTQPPSVSVAPGQTARISCSGDNLGDKYANWYQQKPGQAPVLVIYDDIDRPSGIPERFSGSNSGNTATLTISGTQAEDEADYYCGSYDFFLGLIVFGGGTKLTVL

SEQ ID NO: 30 - protein, 115 aa, Artificial Sequence
  VH of mAb5548
QVQLLESGGGLVQPGGSLRLSCAASGFTFSSYAMSWVRQAPGKGLEWVSTISLTSGFTYYADSVKGRFTISRDNSKNTLYLQMNSLRAEDTAVYYCARQLTLDVWGQGTLVTVSS

SEQ ID NO: 31 - protein, 214 aa, Artificial Sequence
  LC of mAb5548
QSVLTQPPSVSVAPGQTARISCSGDNLGDKYANWYQQKPGQAPVLVIYDDIDRPSGIPERFSGSNSGNTATLTISGTQAEDEADYYCGSYDFFLGLIVFGGGTKLTVLGQPKAAPSVTLFPPSSEELQANKATLVCLISDFYPGAVTVAWKADSSPVKAGVETTTPSKQSNNKYAASSYLSLTPEQWKSHRSYSCQVTHEGSTVEKTVAPTECS

SEQ ID NO: 32 - protein, 445 aa, Artificial Sequence
  HC of mAb5548
QVQLLESGGGLVQPGGSLRLSCAASGFTFSSYAMSWVRQAPGKGLEWVSTISLTSGFTYYADSVKGRFTISRDNSKNTLYLQMNSLRAEDTAVYYCARQLTLDVWGQGTLVTVSSASTKGPSVFPLAPSSKSTSGGTAALGCLVKDYFPEPVTVSWNSGALTSGVHTFPAVLQSSGLYSLSSVVTVPSSSLGTQTYICNVNHKPSNTKVDKKVEPKSCDKTHTCPPCPAPELLGGPSVFLFPPKPKDTLMISRTPEVTCVVVDVSHEDPEVKFNWYVDGVEVHNAKTKPREEQYNSTYRVVSVLTVLHQDWLNGKEYKCKVSNKALPAPIEKTISKAKGQPREPQVYTLPPSRDELTKNQVSLTCLVKGFYPSDIAVEWESNGQPENNYKTTPPVLDSDGSFFLYSKLTVDKSRWQQGNVFSCSVMHEALHNHYTQKSLSLSPGK

SEQ ID NO: 33 - protein, 215 aa, Artificial Sequence
  LC of mAb732
EIVLTQSPATLSLSPGERATLSCRASQNVWAFYLAWYQQKPGQAPRLLIYGASNRATGIPARFSGSGSGTDFTLTISSLEPEDFAVYYCTQYYSSPSLTFGQGTKVEIKGQPKAAPSVTLFPPSSEELQANKATLVCLISDFYPGAVTVAWKADSSPVKAGVETTTPSKQSNNKYAASSYLSLTPEQWKSHRSYSCQVTHEGSTVEKTVAPTECS

SEQ ID NO: 34 - protein, 447 aa, Artificial Sequence
  HC of mAb7024
QVQLVQSGAEVKKPGSSVKVSCKASGGTFSSYAISWVRQAPGQGLEWMGSIIPWFGTTNYAQKFQGRVTITADESTSTAYMELSSLRSEDTAVYYCARDSEYYFDHWGQGTLVTVSSASTKGPSVFPLAPSSKSTSGGTAALGCLVKDYFPEPVTVSWNSGALTSGVHTFPAVLQSSGLYSLSSVVTVPSSSLGTQTYICNVNHKPSNTKVDKKVEPKSCDKTHTCPPCPAPELLGGPSVFLFPPKPKDTLMISRTPEVTCVVVDVSHEDPEVKFNWYVDGVEVHNAKTKPREEQYNSTYRVVSVLTVLHQDWLNGKEYKCKVSNKALPAPIEKTISKAKGQPREPQVYTLPPSRDELTKNQVSLTCLVKGFYPSDIAVEWESNGQPENNYKTTPPVLDSDGSFFLYSKLTVDKSRWQQGNVFSCSVMHEALHNHYTQKSLSLSPGK

SEQ ID NO: 35 - protein, 12 aa, Artificial Sequence
  HCDR3 of mAb3584
EVDSIYYSYFDI

SEQ ID NO: 36 - protein, 123 aa, Artificial Sequence
  VH of mAb3584
QVQLQQSGPGLVKPSQTLSLTCAISGDSVSSSSAAWGWIRQSPRGLEWLGRISYRSKWYNDYAVSVKSRITINPDTSKNQFSLQLNSVTPEDTAVYYCAREVDSIYYSYFDIWGQGTLVTVSS

SEQ ID NO: 37 - protein, 454 aa, Artificial Sequence
  HC of mAb3584
QVQLQQSGPGLVKPSQTLSLTCAISGDSVSSSSAAWGWIRQSPSRGLEWLGRISYRSKWYNDYAVSVKSRITINPDTSKNQFSLQLNSVTPEDTAVYYCAREVDSIYYSYFDIWGQGTLVTVSSASTKGPSVFPLAPSSKSTSGGTAALGCLVKDYFPEPVTVSWNSGALTSGVHTFPAVLQSSGLYSLSSVVTVPSSSLGTQTYICNVNHKPSNTKVDKKVEPKSCDKTHTCPPCPAPELLGGPSVFLFPPKPKDTLMISRTPEVTCVVVDVSHEDPEVKFNWYVDGVEVHNAKTKPREEQYNSTYRVVSVLTVLHQDWLNGKEYKCKVSNKALPAPIEKTISKAKGQPREPQVYTLPPSRDELTKNQVSLTCLVKGFYPSDIAVEWESNGQPENNYKTTPPVLDSDGSFFLYSKLTVDKSRWQQGNVFSCSVMHEALHNHYTQKSLSLSPGK

SEQ ID NO: 38 - protein, 17 aa, Artificial Sequence
  HCDR2 of mAb3077
SIIPWFGWTNYAQKFQG

SEQ ID NO: 39 - protein, 117 aa, Artificial Sequence
  VH of mAb3077
QVQLVQSGAEVKKPGSSVKVSCKASGGTFSSYAISWVRQAPGQGLEWMGSIIPWFGWTNYAQKFQGRVTITADESTSTAYMELSSLRSEDTAVYYCARDSEYYFDHWGQGTLVTVSS